European Patent Specification EP 3 766 518 B1, published January 28, 2026. Title: PCV2 IMMUNOGENIC COMPOSITION FOR LESSENING CLINICAL SYMPTOMS IN PIGS. Applicant: Boehringer Ingelheim Animal Health USA Inc. The sequence listing filed with the application follows.

SEQUENCE LISTING (11 sequences)

SEQ ID NO: 1 - DNA, 8 bp, Artificial
  This is a modified Kozak's sequence
ccgccatg

SEQ ID NO: 2 - DNA, 6 bp, Artificial
  This is a recombinant Eco R1 sequence.
gaattc

SEQ ID NO: 3 - DNA, 713 bp, Porcine circovirus
cagctatgacgtatccaaggaggcgttaccgcagaagaagacaccgcccccgcagccatcttggccagatcctccgccgccgcccctggctcgtccacccccgccaccgctaccgttggagaaggaaaaatggcatcttcaacacccgcctctcccgcaccttcggatatactgtggagaaggaaaaatggcatcttcaacacccgcctctcccgcaccttcggatatactgtgacgactttgttcccccgggaggggggaccaacaaaatctctataccctttgaatactacagaataagaaaggttaaggttgaattctggccctgctcccccatcacccagggtgataggggagtgggctccactgctgttattctagatgataactttgtaacaaaggccacagccctaacctatgacccatatgtaaactactcctcccgccatacaatcccccaacccttctcctaccactcccgttacttcacacccaaacctgttcttgactccactattgattacttccaaccaaataacaaaaggaatcagctttggctgaggctacaaacctctagaaatgtggaccacgtaggcctcggcactgcgttcgaaaacagtaaatacgaccaggactacaatatccgtgtaaccatgtatgtacaattcagagaatttaatcttaaagaccccccacttaaaccctaaatgaat

SEQ ID NO: 4 - DNA, 713 bp, Porcine circovirus
ccgccatgacgtatccaaggaggcgttaccgcagaagaagacaccgcccccgcagccatcttggccagatcctccgccgccgcccctggctcgtccacccccgccaccgctaccgttggagaaggaaaaatggcatcttcaacacccgcctctcccgcaccttcggatatactgtcaaggctaccacagtcacaacgccctcctgggcggtggacatgatgagatttaatattgacgactttgttcccccgggaggggggaccaacaaaatctctataccctttgaatactacagaataagaaaggttaaggttgaattctggccctgctcccccatcacccagggtgataggggagtgggctccactgctgttattctagatgataactttgtaacaaaggccacagccctaacctatgacccatatgtaaactactcctcccgccatacaatcccccaacccttctcctaccactcccgttacttcacacccaaacctgttcttgactccactattgattacttccaaccaaataacaaaaggaatcagctttggctgaggctacaaacctctagaaatgtggaccacgtaggcctcggcactgcgttcgaaaacagtaaatacgaccaggactacaatatccgtgtaaccatgtatgtacaattcagagaatttaatcttaaagaccccccacttgaaccctaagaattc

SEQ ID NO: 5 - protein, 233 aa, Porcine circovirus
MTYPRRRYRRRRHRPRSHLGQILRRRPWLVHPRHRYRWRRKNGIFNTRLSRTFGYTVKATTVTTPSWAVDMMRFNIDDFVPPGGGTNKISIPFEYYRIRKVKVEFWPCSPITQGDRGVGSTAVILDDNFVTKATALTYDPYVNYSSRHTIPQPFSYHSRYFTPKPVLDSTIDYFQPNNKRNQLWLRLQTSRNVDHVGLGTAFENSKYDQDYNIRVTMYVQFREFNLKDPPLKP

SEQ ID NO: 6 - protein, 233 aa, Porcine circovirus
MTYPRRRYRRRRHRPRSHLGQILRRRPWLVHPRHRYRWRRKNGIFNTRLSRTFGYTVKATTVTTPSWAVDMMRFNIDDFVPPGGGTNKISIPFEYYRIRKVKVEFWPCSPITQGDRGVGSTAVILDDNFVTKATALTYDPYVNYSSRHTIPQPFSYHSRYFTPKPVLDSTIDYFQPNNKRNQLWLRLQTSRNVDHVGLGTAFENSKYDQDYNIRVTMYVQFREFNLKDPPLEP

SEQ ID NO: 7 - DNA, 756 bp, Artificial
  This sequence is from porcine circovirus type 2, open reading frame 2, together with a portion from the pGEM T-easy vector.
gcggccgcgggaattcgatccgccatgacgtatccaaggaggcgttaccgcagaagaagacaccgcccccgcagccatcttggccagatcctccgccgccgcccctggctcgtccacccccgccaccgctaccgttggagaaggaaaaatggcatcttcaacacccgcctctcccgcaccttcggatatactgtcaaggctaccacagtcacaacgccctcctgggcggtggacatgatgagatttaatattgacgactttgttcccccgggaggggggaccaacaaaatctctataccctttgaatactacagaataagaaaggttaaggttgaattctggccctgctcccccatcacccagggtgataggggagtgggctccactgctgttattctagatgataactttgtaacaaaggccacagccctaacctatgacccatatgtaaactactcctcccgccatacaatcccccaacccttctcctaccactcccgttacttcacacccaaacctgttcttgactccactattgattacttccaaccaaataacaaaaggaatcagctttggctgaggctacaaacctctagaaatgtggaccacgtaggcctcggcactgcgttcgaaaacagtaaatacgaccaggactacaatatccgtgtaaccatgtatgtacaattcagagaatttaatcttaaagaccccccacttgaaccctaagaattctatcactagtgaattcgcggccgc

SEQ ID NO: 8 - DNA, 10387 bp, Artificial
  This is the porcine circovirus type 2, ORF2 construct, which includes baculovirus and pGEM T-easy coding sequences.
aagctttactcgtaaagcgagttgaaggatcatatttagttgcgtttatgagataagattgaaagcacgtgtaaaatgtttcccgcgcgttggcacaactatttacaatgcggccaagttataaaagattctaatctgatatgttttaaaacacctttgcggcccgagttgtttgcgtacgtgactagcgaagaagatgtgtggaccgcagaacagatagtaaaacaaaaccctagtattggagcaataatcgatttaaccaacacgtctaaatattatgatggtgtgcattttttgcgggcgggcctgttatacaaaaaaattcaagtacctggccagactttgccgcctgaaagcatagttcaagaatttattgacacggtaaaagaatttacagaaaagtgtcccggcatgttggtgggcgtgcactgcacacacggtattaatcgcaccggttacatggtgtgcagatatttaatgcacaccctgggtattgcgccgcaggaagccatagatagattcgaaaaagccagaggtcacaaaattgaaagacaaaattacgttcaagatttattaatttaattaatattatttgcattctttaacaaatactttatcctattttcaaattgttgcgcttcttccagcgaaccaaaactatgcttcgcttgctccgtttagcttgtagccgatcagtggcgttgttccaatcgacggtaggattaggccggatattctccaccacaatgttggcaacgttgatgttacgtttatgcttttggttttccacgtacgtcttttggccggtaatagccgtaaacgtagtgccgtcgcgcgtcacgcacaacaccggatgtttgcgcttgtccgcggggtattgaaccgcgcgatccgacaaatccaccactttggcaactaaatcggtgacctgcgcgtcttttttctgcattatttcgtctttcttttgcatggtttcctggaagccggtgtacatgcggtttagatcagtcatgacgcgcgtgacctgcaaatctttggcctcgatctgcttgtccttgatggcaacgatgcgttcaataaactcttgttttttaacaagttcctcggttttttgcgccaccaccgcttgcagcgcgtttgtgtgctcggtgaatgtcgcaatcagcttagtcaccaactgtttgctctcctcctcccgttgtttgatcgcgggatcgtacttgccggtgcagagcacttgaggaattacttcttctaaaagccattcttgtaattctatggcgtaaggcaatttggacttcataatcagctgaatcacgccggatttagtaatgagcactgtatgcggctgcaaatacagcgggtcgccccttttcacgacgctgttagaggtagggcccccattttggatggtctgctcaaataacgatttgtatttattgtctacatgaacacgtatagctttatcacaaactgtatattttaaactgttagcgacgtccttggccacgaaccggacctgttggtcgcgctctagcacgtaccgcaggttgaacgtatcttctccaaatttaaattctccaattttaacgcgagccattttgatacacgtgtgtcgattttgcaacaactattgttttttaacgcaaactaaacttattgtggtaagcaataattaaatatgggggaacatgcgccgctacaacactcgtcgttatgaacgcagacggcgccggtctcggcgcaagcggctaaaacgtgttgcgcgttcaacgcggcaaacatcgcaaaagccaatagtacagttttgatttgcatattaacggcgattttttaaattatcttatttaataaatagttatgacgcctacaactccccgcccgcgttgactcgctgcacctcgagcagttcgttgacgccttcctccgtgtggccgaacacgtcgagcgggtggtcgatgaccagcggcgtgccgcacgcgacgcacaagtatctgtacaccgaatgatcgtcgggcgaaggcacgtcggcctccaagtggcaatattggcaaattcgaaaatatatacagttgggttgtttgcgcatatctatcgtggcgttgggcatgtacgtccgaacgttgatttgcatgcaagccgaaattaaatcattgcgattagtgcgattaaaacgttgtacatcctcgcttttaatcatgccgtcgattaaatcgcgcaatcgagtcaagtgatcaaagtgtggaataatgttttctttgtattcccgagtcaagcgcagcgcgtattttaacaaactagccatcttgtaagttagtttcatttaatgcaactttatccaataatatattatgtatcgcacgtcaagaattaacaatgcgcccgttgtcgcatctcaacacgactatgatagagatcaaataaagcgcgaattaaatagcttgcgacgcaacgtgcacgatctgtgcacgcgttccggcacgagctttgattgtaataagtttttacgaagcgatgacatgacccccgtagtgacaacgatcacgcccaaaagaactgccgactacaaaattaccgagtatgtcggtgacgttaaaactattaagccatccaatcgaccgttagtcgaatcaggaccgctggtgcgagaagccgcgaagtatggcgaatgcatcgtataacgtgtggagtccgctcattagagcgtcatgtttagacaagaaagctacatatttaattgatcccgatgattttattgataaattgaccctaactccatacacggtattctacaatggcggggttttggtcaaaatttccggactgcgattgtacatgctgttaacggctccgcccactattaatgaaattaaaaattccaattttaaaaaacgcagcaagagaaacatttgtatgaaagaatgcgtagaaggaaagaaaaatgtcgtcgacatgctgaacaacaagattaatatgcctccgtgtataaaaaaaatattgaacgatttgaaagaaaacaatgtaccgcgcggcggtatgtacaggaagaggtttatactaaactgttacattgcaaacgtggtttcgtgtgccaagtgtgaaaaccgatgtttaatcaaggctctgacgcatttctacaaccacgactccaagtgtgtgggtgaagtcatgcatcttttaatcaaatcccaagatgtgtataaaccaccaaactgccaaaaaatgaaaactgtcgacaagctctgtccgtttgctggcaactgcaagggtctcaatcctatttgtaattattgaataataaaacaattataaatgctaaatttgttttttattaacgatacaaaccaaacgcaacaagaacatttgtagtattatctataattgaaaacgcgtagttataatcgctgaggtaatatttaaaatcattttcaaatgattcacagttaatttgcgacaatataattttattttcacataaactagacgccttgtcgtcttcttcttcgtattccttctctttttcatttttctcctcataaaaattaacatagttattatcgtatccatatatgtatctatcgtatagagtaaattttttgttgtcataaatatatatgtcttttttaatggggtgtatagtaccgctgcgcatagtttttctgtaatttacaacagtgctattttctggtagttcttcggagtgtgttgctttaattattaaatttatataatcaatgaatttgggatcgtcggttttgtacaatatgttgccggcatagtacgcagcttcttctagttcaattacaccattttttagcagcaccggattaacataactttccaaaatgttgtacgaaccgttaaacaaaaacagttcacctcccttttctatactattgtctgcgagcagttgtttgttgttaaaaataacagccattgtaatgagacgcacaaactaatatcacaaactggaaatgtctatcaatatatagttgctgatatcatggagataattaaaatgataaccatctcgcaaataaataagtattttactgttttcgtaacagttttgtaataaaaaaacctataaatattccggattattcataccgtcccaccatcgggcgcggatcagatctgcagcggccgcgggaattcgatccgccatgacgtatccaaggaggcgttaccgcagaagaagacaccgcccccgcagccatcttggccagatcctccgccgccgcccctggctcgtccacccccgccaccgctaccgttggagaaggaaaaatggcatcttcaacacccgcctctcccgcaccttcggatatactgtcaaggctaccacagtcacaacgccctcctgggcggtggacatgatgagatttaatattgacgactttgttcccccgggaggggggaccaacaaaatctctataccctttgaatactacagaataagaaaggttaaggttgaattctggccctgctcccccatcacccagggtgataggggagtgggctccactgctgttattctagatgataactttgtaacaaaggccacagccctaacctatgacccatatgtaaactactcctcccgccatacaatcccccaacccttctcctaccactcccgttacttcacacccaaacctgttcttgactccactattgattacttccaaccaaataacaaaaggaatcagctttggctgaggctacaaacctctagaaatgtggaccacgtaggcctcggcactgcgttcgaaaacagtaaatacgaccaggactacaatatccgtgtaaccatgtatgtacaattcagagaatttaatcttaaagaccccccacttgaaccctaagaattctatcactagtgaattcgcggccgccggccgctccagaattctagaaggtacccgggatcctttcctgggacccggcaagaaccaaaaactcactctcttcaaggaaatccgtaatgttaaacccgacacgatgaagcttgtcgttggatggaaaggaaaagagttctacagggaaacttggacccgcttcatggaagacagcttccccattgttaacgaccaagaagtgatggatgttttccttgttgtcaacatgcgtcccactagacccaaccgttgttacaaattcctggcccaacacgctctgcgttgcgaccccgactatgtacctcatgacgtgattaggatcgtcgagccttcatgggtgggcagcaacaacgagtaccgcatcagcctggctaagaagggcggcggctgcccaataatgaaccttcactctgagtacaccaactcgttcgaacagttcatcgatcgtgtcatctgggagaacttctacaagcccatcgtttacatcggtaccgactctgctgaagaggaggaaattctccttgaagtttccctggtgttcaaagtaaaggagtttgcaccagacgcacctctgttcactggtccggcgtattaaaacacgatacattgttattagtacatttattaagcgctagattctgtgcgttgttgatttacagacaattgttgtacgtattttaataattcattaaatttataatctttagggtggtatgttagagcgaaaatcaaatgattttcagcgtctttatatctgaatttaaatattaaatcctcaatagatttgtaaaataggtttcgattagtttcaaacaagggttgtttttccgaaccgatggctggactatctaatggattttcgctcaacgccacaaaacttgccaaatcttgtagcagcaatctagctttgtcgatattcgtttgtgttttgttttgtaataaaggttcgacgtcgttcaaaatattatgcgcttttgtatttctttcatcactgtcgttagtgtacaattgactcgacgtaaacacgttaaataaagcttggacatatttaacatcgggcgtgttagctttattaggccgattatcgtcgtcgtcccaaccctcgtcgttagaagttgcttccgaagacgattttgccatagccacacgacgcctattaattgtgtcggctaacacgtccgcgatcaaatttgtagttgagctttttggaattatttctgattgcgggcgtttttgggcgggtttcaatctaactgtgcccgattttaattcagacaacacgttagaaagcgatggtgcaggcggtggtaacatttcagacggcaaatctactaatggcggcggtggtggagctgatgataaatctaccatcggtggaggcgcaggcggggctggcggcggaggcggaggcggaggtggtggcggtgatgcagacggcggtttaggctcaaatgtctctttaggcaacacagtcggcacctcaactattgtactggtttcgggcgccgtttttggtttgaccggtctgagacgagtgcgatttttttcgtttctaatagcttccaacaattgttgtctgtcgtctaaaggtgcagcgggttgaggttccgtcggcattggtggagcgggcggcaattcagacatcgatggtggtggtggtggtggaggcgctggaatgttaggcacgggagaaggtggtggcggcggtgccgccggtataatttgttctggtttagtttgttcgcgcacgattgtgggcaccggcgcaggcgccgctggctgcacaacggaaggtcgtctgcttcgaggcagcgcttggggtggtggcaattcaatattataattggaatacaaatcgtaaaaatctgctataagcattgtaatttcgctatcgtttaccgtgccgatatttaacaaccgctcaatgtaagcaattgtattgtaaagagattgtctcaagctcgccgcacgccgataacaagccttttcatttttactacagcattgtagtggcgagacacttcgctgtcgtcgacgtacatgtatgctttgttgtcaaaaacgtcgttggcaagctttaaaatatttaaaagaacatctctgttcagcaccactgtgttgtcgtaaatgttgtttttgataatttgcgcttccgcagtatcgacacgttcaaaaaattgatgcgcatcaattttgttgttcctattattgaataaataagattgtacagattcatatctacgattcgtcatggccaccacaaatgctacgctgcaaacgctggtacaattttacgaaaactgcaaaaacgtcaaaactcggtataaaataatcaacgggcgctttggcaaaatatctattttatcgcacaagcccactagcaaattgtatttgcagaaaacaatttcggcgcacaattttaacgctgacgaaataaaagttcaccagttaatgagcgaccacccaaattttataaaaatctattttaatcacggttccatcaacaaccaagtgatcgtgatggactacattgactgtcccgatttatttgaaacactacaaattaaaggcgagctttcgtaccaacttgttagcaatattattagacagctgtgtgaagcgctcaacgatttgcacaagcacaatttcatacacaacgacataaaactcgaaaatgtcttatatttcgaagcacttgatcgcgtgtatgtttgcgattacggattgtgcaaacacgaaaactcacttagcgtgcacgacggcacgttggagtattttagtccggaaaaaattcgacacacaactatgcacgtttcgtttgactggtacgcggcgtgttaacatacaagttgctaacgtaatcatggtcatagctgtttcctgtgtgaaattgttatccgctcacaattccacacaacatacgagccggaagcataaagtgtaaagcctggggtgcctaatgagtgagctaactcacattaattgcgttgcgctcactgcccgctttccagtcgggaaacctgtcgtgccagctgcattaatgaatcggccaacgcgcggggagaggcggtttgcgtattgggcgctcttccgcttcctcgctcactgactcgctgcgctcggtcgttcggctgcggcgagcggtatcagctcactcaaaggcggtaatacggttatccacagaatcaggggataacgcaggaaagaacatgtgagcaaaaggccagcaaaaggccaggaaccgtaaaaaggccgcgttgctggcgtttttccataggctccgcccccctgacgagcatcacaaaaatcgacgctcaagtcagaggtggcgaaacccgacaggactataaagataccaggcgtttccccctggaagctccctcgtgcgctctcctgttccgaccctgccgcttaccggatacctgtccgcctttctcccttcgggaagcgtggcgctttctcatagctcacgctgtaggtatctcagttcggtgtaggtcgttcgctccaagctgggctgtgtgcacgaaccccccgttcagcccgaccgctgcgccttatccggtaactatcgtcttgagtccaacccggtaagacacgacttatcgccactggcagcagccactggtaacaggattagcagagcgaggtatgtaggcggtgctacagagttcttgaagtggtggcctaactacggctacactagaaggacagtatttggtatctgcgctctgctgaagccagttaccttcggaaaaagagttggtagctcttgatccggcaaacaaaccaccgctggtagcggtggtttttttgtttgcaagcagcagattacgcgcagaaaaaaaggatctcaagaagatcctttgatcttttctacggggtctgacgctcagtggaacgaaaactcacgttaagggattttggtcatgagattatcaaaaaggatcttcacctagatccttttaaattaaaaatgaagttttaaatcaatctaaagtatatatgagtaaacttggtctgacagttaccaatgcttaatcagtgaggcacctatctcagcgatctgtctatttcgttcatccatagttgcctgactccccgtcgtgtagataactacgatacgggagggcttaccatctggccccagtgctgcaatgataccgcgagacccacgctcaccggctccagatttatcagcaataaaccagccagccggaagggccgagcgcagaagtggtcctgcaactttatccgcctccatccagtctattaattgttgccgggaagctagagtaagtagttcgccagttaatagtttgcgcaacgttgttgccattgctacaggcatcgtggtgtcacgctcgtcgtttggtatggcttcattcagctccggttcccaacgatcaaggcgagttacatgatcccccatgttgtgcaaaaaagcggttagctccttcggtcctccgatcgttgtcagaagtaagttggccgcagtgttatcactcatggttatggcagcactgcataattctcttactgtcatgccatccgtaagatgcttttctgtgactggtgagtactcaaccaagtcattctgagaatagtgtatgcggcgaccgagttgctcttgcccggcgtcaatacgggataataccgcgccacatagcagaactttaaaagtgctcatcattggaaaacgttcttcggggcgaaaactctcaaggatcttaccgctgttgagatccagttcgatgtaacccactcgtgcacccaactgatcttcagcatcttttactttcaccagcgtttctgggtgagcaaaaacaggaaggcaaaatgccgcaaaaaagggaataagggcgacacggaaatgttgaatactcatactcttcctttttcaatattattgaagcatttatcagggttattgtctcatgagcggatacatatttgaatgtatttagaaaaataaacaaataggggttccgcgcacatttccccgaaaagtgccacctgacgtctaagaaaccattattatcatgacattaacctataaaaataggcgtatcacgaggccctttcgtctcgcgcgtttcggtgatgacggtgaaaacctctgacacatgcagctcccggagacggtcacagcttgtctgtaagcggatgccgggagcagacaagcccgtcagggcgcgtcagcgggtgttggcgggtgtcggggctggcttaactatgcggcatcagagcagattgtactgagagtgcaccatatgcggtgtgaaataccgcacagatgcgtaaggagaaaataccgcatcaggcgccattcgccattcaggctgcgcaactgttgggaagggcgatcggtgcgggcctcttcgctattacgccagctggcgaaagggggatgtgctgcaaggcgattaagttgggtaacgccagggttttcccagtcacgacgttgtaaaacgacggccagtgcc

SEQ ID NO: 9 - protein, 20 aa, Porcine circovirus
SYPRRRYRRRRHHPPSHLGQ

SEQ ID NO: 10 - protein, 19 aa, Porcine circovirus
PRHHYRPRRKNGIFNTTLS

SEQ ID NO: 11 - protein, 233 aa, Artificial
  This is an amino acid sequence for porcine circovirus type 2, open reading frame 2.
MTYPRRRYRRRRHRPRSHLGQILRRRPWLVHPRHRYRWRRKNGIFNTRLSRTFGYTVKATTVRTPSWAVDMMRFNIDDFVPPGGGTNKISIPFEYYRIKKVKVEFWPCSPITQGDRGVGSTAVILDDNFVTKATALTYDPYVNYSSRHTIPQPFSYHSRYFTPKPVLDSTIDYFQPNNKRNQLWLRLQTSRNVDHVGLGTAFENSIYDQDYNIRVTMYVQFREFNLKDPPLKP